European Patent Specification EP 2 730 663 B1, published March 22, 2023. Title: Genetic factors associated with inhibitor development in hemophilia A. Applicant: Erik Berntorp Jan Astermark. The sequence listing filed with the application follows.

SEQUENCE LISTING (1 sequence)

SEQ ID NO: 1 - DNA, 52 bp, homo sapiens
  purine (27)..(27): nucleotide r can be g or a
ttgccactacttgtctccaaagaaacrtaagaatgctttatcatacaacagt